European Patent Application EP 4 745 161 A2, published May 20, 2026. Title: Antibodies for the treatment of ErbB-2/ErbB-3 positive tumors. Applicant: Merus N.V. Application EP. The sequence listing filed with the application follows.

SEQUENCE LISTING (141 sequences)

SEQ ID NO: 1 - DNA, 370 bp, synthetic construct
  misc_feature 1..370: note = MF2926
  source 1..370: mol_type = other DNA
  CDS 20..370
ggcccagccggccatggcccaggtccagctgcagcagtctggacctgagctggtgaaacctggggcttcagtgatgatttcctgcaaggcttctggttactcattcactggctaccacatgaactgggtgaagcaaagtcctgaaaagagccttgagtggattggagacataaatcctagcattggtacgactgcccacaaccagattttcagggccaaggccacaatgactgttgacaaatcctccaacacagcctacatgcagctcaagagcctgacatctgaagactctggagtcttttactgtgttagaagaggggactggtccttcgatgtctggggcacagggaccacggtcaccgtctccagt

SEQ ID NO: 2 - protein, 117 aa, synthetic construct
  REGION 1..117: note = Synthetic Construct; note = translation of SEQ ID NO:1
QVQLQQSGPELVKPGASVMISCKASGYSFTGYHMNWVKQSPEKSLEWIGDINPSIGTTAHNQIFRAKATMTVDKSSNTAYMQLKSLTSEDSGVFYCVRRGDWSFDVWGTGTTVTVSS

SEQ ID NO: 3 - protein, 16 aa, synthetic construct
  REGION 1..16: note = MF2926 CDR1
GYHMNWVKQSPEKSLE

SEQ ID NO: 4 - protein, 6 aa, synthetic construct
  REGION 1..6: note = MF2926 CDR2
NQIFRA

SEQ ID NO: 5 - protein, 8 aa, synthetic construct
  REGION 1..8: note = MF2926 CDR3
RGDWSFDV

SEQ ID NO: 6 - DNA, 379 bp, synthetic construct
  misc_feature 1..379: note = MF2930
  source 1..379: mol_type = other DNA
  CDS 20..379
ggcccagccggccatggccgaggtccagctgcagcagtctggggctgaactggtgaagcctggagcctcagtgatgatgtcctgtaaggtttctggctacaccttcacttcctatcctatagcgtggatgaagcaggttcatggaaagagcctagagtggattggaaattttcatccttacagtgatgatactaagtacaatgaaaacttcaagggcaaggccacattgactgtagaaaaatcctctagcacagtctacttggagctcagccgattaacatctgatgactctgctgtttattactgtgcaagaagtaacccattatattactttgctatggactactggggtcaaggaacctcggtcaccgtctccagt

SEQ ID NO: 7 - protein, 120 aa, synthetic construct
  REGION 1..120: note = Synthetic Construct; note = translation of SEQ ID NO:6
EVQLQQSGAELVKPGASVMMSCKVSGYTFTSYPIAWMKQVHGKSLEWIGNFHPYSDDTKYNENFKGKATLTVEKSSSTVYLELSRLTSDDSAVYYCARSNPLYYFAMDYWGQGTSVTVSS

SEQ ID NO: 8 - protein, 16 aa, synthetic construct
  REGION 1..16: note = MF2930 CDR1
SYPIAWMKQVHGKSLE

SEQ ID NO: 9 - protein, 6 aa, synthetic construct
  REGION 1..6: note = MF2930 CDR2
NENFKG

SEQ ID NO: 10 - protein, 11 aa, synthetic construct
  REGION 1..11: note = MF2930 CDR3
SNPLYYFAMDY

SEQ ID NO: 11 - DNA, 385 bp, synthetic construct
  misc_feature 1..385: note = MF1849
  source 1..385: mol_type = other DNA
  CDS 20..385
ggcccagccggccatggcccaggtgcagctggtggagtctgggggaggcgtggtccagcctgggaggtccctgagactctcctgtgcagcctctggattcaccttcagtagctatggcatgcactgggtccgccaggctccaggcaaggggctggagtgggtggcagttatatcatatgatggaagtaataaatactatgcagactccgtgaagggccgattcaccatctccagagacaattccaagaacacgctgtatctgcaaatgaacagcctgagagctgaggacacggccgtgtattactgtgcaaaaggtgactacggttcttactcttcttacgcctttgattattggggccaaggtaccctggtcaccgtctccagt

SEQ ID NO: 12 - protein, 122 aa, synthetic construct
  REGION 1..122: note = Synthetic Construct; note = translation of SEQ ID NO:11
QVQLVESGGGVVQPGRSLRLSCAASGFTFSSYGMHWVRQAPGKGLEWVAVISYDGSNKYYADSVKGRFTISRDNSKNTLYLQMNSLRAEDTAVYYCAKGDYGSYSSYAFDYWGQGTLVTVSS

SEQ ID NO: 13 - protein, 5 aa, synthetic construct
  REGION 1..5: note = MF1849 CDR1
SYGMH

SEQ ID NO: 14 - protein, 17 aa, synthetic construct
  REGION 1..17: note = MF1849 CDR2
VISYDGSNKYYADSVKG

SEQ ID NO: 15 - protein, 13 aa, synthetic construct
  REGION 1..13: note = MF1849 CDR3
GDYGSYSSYAFDY

SEQ ID NO: 16 - DNA, 385 bp, synthetic construct
  misc_feature 1..385: note = MF2973
  source 1..385: mol_type = other DNA
  CDS 20..385
ggcccagccggccatggcccaggtgcagctgaagcagtctggggctgagctggtgaggcctggggcttcagtgaagttgtcctgcaaggcttctggctacattttcactggctactatataaactggttgaggcagaggcctggacagggacttgaatggattgcaaaaatttatcctggaagtggtaatacttactacaatgagaagttcaggggcaaggccacactgactgcagaagaatcctccagcactgcctacatgcagctcagcagcctgacatctgaggactctgctgtctatttctgtgcaagagggccccactatgattacgacggcccctggtttgtttactggggccaagggactctggtcaccgtctccagt

SEQ ID NO: 17 - protein, 122 aa, synthetic construct
  REGION 1..122: note = Synthetic Construct; note = translation of SEQ ID NO:16
QVQLKQSGAELVRPGASVKLSCKASGYIFTGYYINWLRQRPGQGLEWIAKIYPGSGNTYYNEKFRGKATLTAEESSSTAYMQLSSLTSEDSAVYFCARGPHYDYDGPWFVYWGQGTLVTVSS

SEQ ID NO: 18 - protein, 16 aa, synthetic construct
  REGION 1..16: note = MF2973 CDR1
GYYINWLRQRPGQGLE

SEQ ID NO: 19 - protein, 6 aa, synthetic construct
  REGION 1..6: note = MF2973 CDR2
NEKFRG

SEQ ID NO: 20 - protein, 13 aa, synthetic construct
  REGION 1..13: note = MF2973 CDR3
GPHYDYDGPWFVY

SEQ ID NO: 21 - DNA, 382 bp, synthetic construct
  misc_feature 1..382: note = MF3004
  source 1..382: mol_type = other DNA
  CDS 20..382
ggcccagccggccatggcccaggtgcagctgaagcagtctggggctgagctggtgaggcctggggcttcagtgaagctgtcctgcaaggcttctggctacactttcactggctactatataaactgggtgaagcagaggcctggacagggacttgagtggattgcaaggatttatcctggaagtggttatacttactacaatgagaagttcaagggcaaggccacactgactgcagaagaatcctccagcactgcctacatgcacctcagcagcctgacatctgaggactctgctgtctatttctgtgcaagaccccactatggttacgacgactggtacttcggtgtctggggcacaggcaccacggtcaccgtctccagt

SEQ ID NO: 22 - protein, 121 aa, synthetic construct
  REGION 1..121: note = Synthetic Construct; note = translation of SEQ ID NO:21
QVQLKQSGAELVRPGASVKLSCKASGYTFTGYYINWVKQRPGQGLEWIARIYPGSGYTYYNEKFKGKATLTAEESSSTAYMHLSSLTSEDSAVYFCARPHYGYDDWYFGVWGTGTTVTVSS

SEQ ID NO: 23 - protein, 16 aa, synthetic construct
  REGION 1..16: note = MF3004 CDR1
GYYINWVKQRPGQGLE

SEQ ID NO: 24 - protein, 6 aa, synthetic construct
  REGION 1..6: note = MF3004 CDR2
NEKFKG

SEQ ID NO: 25 - protein, 12 aa, synthetic construct
  REGION 1..12: note = MF3004 CDR3
PHYGYDDWYFGV

SEQ ID NO: 26 - DNA, 382 bp, synthetic construct
  misc_feature 1..382: note = MF2971
  source 1..382: mol_type = other DNA
ggcccagccggccatggcccaggtgcagctgaagcagtctggggctgagctggtgaggcctggggcttcagtgaaactgtcctgcaaggcttctggctacactttcactgcctactatataaactgggtgaagcagaggcctggacagggacttgagtggattgcaaggatttatcctggaagtggctatacttactacaatgagattttcaagggcagggccacactgactgcagacgaatcctccagcactgcctacatgcaactcagcagcctgacatctgaggactctgctgtctatttctgtgcaagacctccggtctactatgactcggcctggtttgcttactggggccaagggactctggtcaccgtctccagt

SEQ ID NO: 27 - protein, 16 aa, synthetic construct
  REGION 1..16: note = MF2971 CDR1
AYYINWVKQRPGQGLE

SEQ ID NO: 28 - protein, 6 aa, synthetic construct
  REGION 1..6: note = MF2971 CDR2
NEIFKG

SEQ ID NO: 29 - protein, 12 aa, synthetic construct
  REGION 1..12: note = MF2971 CDR3
PPVYYDSAWFAY

SEQ ID NO: 30 - DNA, 382 bp, synthetic construct
  misc_feature 1..382: note = MF3025
  source 1..382: mol_type = other DNA
  CDS 20..382
ggcccagccggccatggcccaggtgcagctgaagcagtctggggctgagctggtgaggcctgggacttcagtgaagctgtcctgcaaggcttctggctacactttcactggctactatataaactgggtgaagcagaggcctggacagggacttgagtggattgcaaggatttatcctggaagtggttatacttactacaatgagaagttcaagggcaaggccacactgactgcagaagaatcctccaacactgcctatatgcacctcagcagcctgacatctgaggactctgctgtctatttctgtgcaaggccccactatggttacgacgactggtacttcgctgtctggggcacagggaccacggtcaccgtctccagt

SEQ ID NO: 31 - protein, 121 aa, synthetic construct
  REGION 1..121: note = Synthetic Construct; note = translation of SEQ ID NO:30
QVQLKQSGAELVRPGTSVKLSCKASGYTFTGYYINWVKQRPGQGLEWIARIYPGSGYTYYNEKFKGKATLTAEESSNTAYMHLSSLTSEDSAVYFCARPHYGYDDWYFAVWGTGTTVTVSS

SEQ ID NO: 32 - protein, 16 aa, synthetic construct
  REGION 1..16: note = MF3025 CDR1
GYYINWVKQRPGQGLE

SEQ ID NO: 33 - protein, 6 aa, synthetic construct
  REGION 1..6: note = MF3025 CDR2
NEKFKG

SEQ ID NO: 34 - protein, 12 aa, synthetic construct
  REGION 1..12: note = MF3025 CDR3
PHYGYDDWYFAV

SEQ ID NO: 35 - DNA, 385 bp, synthetic construct
  misc_feature 1..385: note = MF2916
  source 1..385: mol_type = other DNA
  CDS 20..385
ggcccagccggccatggcccaggtccagctgcagcagtctggggctgagctggtgaggcctggggcttcagtgaagctgtcctgcaaggcttctggctacactttcactggctactatataaactgggtgaagcagaggcctggacagggacttgagtggattgcaaggatttatcctggcagtggtcatacttcctacaatgagaagttcaagggcaaggccacactgactacagaaaaatcctccagcactgcctacatgcagctcagcagcctgacatctgaggactctgctgtctatttctgtgcaagacctatctactttgattacgcaggggggtacttcgatgtctggggcacaagaacctcggtcaccgtctccagt

SEQ ID NO: 36 - protein, 122 aa, synthetic construct
  REGION 1..122: note = Synthetic Construct; note = translation of SEQ ID NO:35
QVQLQQSGAELVRPGASVKLSCKASGYTFTGYYINWVKQRPGQGLEWIARIYPGSGHTSYNEKFKGKATLTTEKSSSTAYMQLSSLTSEDSAVYFCARPIYFDYAGGYFDVWGTRTSVTVSS

SEQ ID NO: 37 - protein, 13 aa, synthetic construct
  REGION 1..13: note = MF2916 CDR3
PIYFDYAGGYFDV

SEQ ID NO: 38 - DNA, 382 bp, synthetic construct
  misc_feature 1..382: note = MF3958
  source 1..382: mol_type = other DNA
  CDS 20..382
ggcccagccggccatggcccaggtgcagctggtgcagtctggcgccgaagtgaagaaacctggcgccagcgtgaagctgagctgcaaggccagcggctacaccttcaccgcctactacatcaactgggtccgacaggccccaggccagggcctggaatggatcggcagaatctaccccggctccggctacaccagctacgcccagaagttccagggcagagccaccctgaccgccgacgagagcaccagcaccgcctacatggaactgagcagcctgcggagcgaggataccgccgtgtacttctgcgccagaccccccgtgtactacgacagcgcttggtttgcctactggggccagggcaccctggtcaccgtctccagt

SEQ ID NO: 39 - protein, 121 aa, synthetic construct
  REGION 1..121: note = Synthetic Construct; note = translation of SEQ ID NO:38
QVQLVQSGAEVKKPGASVKLSCKASGYTFTAYYINWVRQAPGQGLEWIGRIYPGSGYTSYAQKFQGRATLTADESTSTAYMELSSLRSEDTAVYFCARPPVYYDSAWFAYWGQGTLVTVSS

SEQ ID NO: 40 - protein, 5 aa, synthetic construct
  REGION 1..5: note = MF3958 CDR1
AYYIN

SEQ ID NO: 41 - protein, 17 aa, synthetic construct
  REGION 1..17: note = MF3958 CDR2
RIYPGSGYTSYAQKFQG

SEQ ID NO: 42 - protein, 12 aa, synthetic construct
  REGION 1..12: note = MF3958 CDR3
PPVYYDSAWFAY

SEQ ID NO: 43 - DNA, 382 bp, synthetic construct
  misc_feature 1..382: note = MF3031
  source 1..382: mol_type = other DNA
ggcccagccggccatggcccaggtccagctgcagcagtctggggctgagctggtgaggcctggggcttcagtgaagctgtcctgcaaggcttctggctacactttcactgcctactatataaactgggtgaagcagaggcctggacagggacttgagtggattgcaaagatttatcctggaagtggttatacttactacaatgagaatttcaggggcaaggccacactgactgcagaagaatcctccagtactgcctacatacaactcagcagcctgacatctgaggactctgctgtctatttctgtgcaagaggcgtctatgattacgacggggcctggtttgcttactggggccaagggactctggtcaccgtctccagt

SEQ ID NO: 44 - protein, 16 aa, synthetic construct
  REGION 1..16: note = MF3031 CDR1
AYYINWVKQRPGQGLE

SEQ ID NO: 45 - protein, 6 aa, synthetic construct
  REGION 1..6: note = MF3031 CDR2
NENFRG

SEQ ID NO: 46 - protein, 12 aa, synthetic construct
  REGION 1..12: note = MF3031 CDR3
GVYDYDGAWFAY

SEQ ID NO: 47 - DNA, 382 bp, synthetic construct
  misc_feature 1..382: note = MF3991
  source 1..382: mol_type = other DNA
  CDS 20..382
ggcccagccggccatggcccaggtgcagctggtgcagtctggcgccgaagtgaagaaacctggcgccagcgtgaagctgagctgcaaggccagcggctacaccttcaccgcctactacatcaactgggtccgacaggccccaggccagggcctggaatggatcggcagaatctaccccggctccggctacaccagctacgcccagaagttccagggcagagccaccctgaccgccgacgagagcaccagcaccgcctacatggaactgagcagcctgcggagcgaggataccgccgtgtacttctgcgccagaccccactacggctacgacgactggtacttcggcgtgtggggccagggcaccctggtcaccgtctccagt

SEQ ID NO: 48 - protein, 121 aa, synthetic construct
  REGION 1..121: note = Synthetic Construct; note = translation of SEQ ID NO:47
QVQLVQSGAEVKKPGASVKLSCKASGYTFTAYYINWVRQAPGQGLEWIGRIYPGSGYTSYAQKFQGRATLTADESTSTAYMELSSLRSEDTAVYFCARPHYGYDDWYFGVWGQGTLVTVSS

SEQ ID NO: 49 - protein, 5 aa, synthetic construct
  REGION 1..5: note = MF3991 CDR1
AYYIN

SEQ ID NO: 50 - protein, 17 aa, synthetic construct
  REGION 1..17: note = MF3991 CDR2
RIYPGSGYTSYAQKFQG

SEQ ID NO: 51 - protein, 12 aa, synthetic construct
  REGION 1..12: note = MF3991 CDR3
PHYGYDDWYFGV

SEQ ID NO: 52 - DNA, 391 bp, synthetic construct
  misc_feature 1..391: note = MF3178
  source 1..391: mol_type = other DNA
  CDS 20..391
ggcccagccggccatggcccaggtgcagctggtgcagtctggggctgaggtgaagaagcctggggcctcagtgaaggtctcctgcaaggcttctggatacaccttcaccggctactatatgcactgggtgcgacaggcccctggacaagggcttgagtggatgggatggatcaaccctaacagtggtggcacaaactatgcacagaagtttcagggcagggtcacgatgaccagggacacgtccatcagcacagcctacatggagctgagcaggctgagatctgacgacacggctgtgtattactgtgcaagagatcatggttctcgtcatttctggtcttactggggctttgattattggggccaaggtaccctggtcaccgtctccagt

SEQ ID NO: 53 - protein, 124 aa, synthetic construct
  REGION 1..124: note = Synthetic Construct; note = translation of SEQ ID NO:52
QVQLVQSGAEVKKPGASVKVSCKASGYTFTGYYMHWVRQAPGQGLEWMGWINPNSGGTNYAQKFQGRVTMTRDTSISTAYMELSRLRSDDTAVYYCARDHGSRHFWSYWGFDYWGQGTLVTVSS

SEQ ID NO: 54 - protein, 5 aa, synthetic construct
  REGION 1..5: note = MF3178 CDR1
GYYMH

SEQ ID NO: 55 - protein, 17 aa, synthetic construct
  REGION 1..17: note = MF3178 CDR2
WINPNSGGTNYAQKFQG

SEQ ID NO: 56 - protein, 15 aa, synthetic construct
  REGION 1..15: note = MF3178 CDR3
DHGSRHFWSYWGFDY

SEQ ID NO: 57 - DNA, 385 bp, synthetic construct
  misc_feature 1..385: note = MF3176
  source 1..385: mol_type = other DNA
  CDS 20..385
ggcccagccggccatggccgaggtgcagctgttggagtctgggggaggcttggtacagcctggggggtccctgagactctcctgtgcagcctctggattcacctttagcagctatgccatgagctgggtccgccaggctccagggaaggggctggagtgggtctcagctattagtggtagtggtggtagcacatactacgcagactccgtgaagggccggttcaccatctccagagacaattccaagaacacgctgtatctgcaaatgaacagcctgagagccgaggacacggctgtgtattactgtgcaagagattggtggtacccgccgtactactggggctttgattattggggccaaggtaccctggtcaccgtctccagt

SEQ ID NO: 58 - protein, 122 aa, synthetic construct
  REGION 1..122: note = Synthetic Construct; note = translation of SEQ ID NO:57
EVQLLESGGGLVQPGGSLRLSCAASGFTFSSYAMSWVRQAPGKGLEWVSAISGSGGSTYYADSVKGRFTISRDNSKNTLYLQMNSLRAEDTAVYYCARDWWYPPYYWGFDYWGQGTLVTVSS

SEQ ID NO: 59 - protein, 5 aa, synthetic construct
  REGION 1..5: note = MF3176 CDR1
SYAMS

SEQ ID NO: 60 - protein, 17 aa, synthetic construct
  REGION 1..17: note = MF3176 CDR2
AISGSGGSTYYADSVKG

SEQ ID NO: 61 - protein, 13 aa, synthetic construct
  REGION 1..13: note = MF3176 CDR3
DWWYPPYYWGFDY

SEQ ID NO: 62 - DNA, 391 bp, synthetic construct
  misc_feature 1..391: note = MF3163
  source 1..391: mol_type = other DNA
ggcccagccggccatggcccaggtgcagctggtgcagtctggggctgaggtgaagaagcctggggcctcagtgaaggtctcctgcaaggcttctggatacaccttcaccggctactatatgcactgggtgcgacaggcccctggacaagggcttgagtggatgggatggatcaaccctaacagtggtggcacaaactatgcacagaagtttcagggcagggtcacgatgaccagggacacgtccatcagcacagcctacatggagctgagcaggctgagatctgacgacacggccgtgtattactgtgcaaaagattcttactctcgtcatttctactcttggtgggcctttgattattggggccaaggtaccctggtcaccgtctccagt

SEQ ID NO: 63 - protein, 17 aa, synthetic construct
  REGION 1..17: note = MF3163 CDR2
WINPNSGGTNYAQKFQG

SEQ ID NO: 64 - protein, 15 aa, synthetic construct
  REGION 1..15: note = MF3163 CDR3
DSYSRHFYSWWAFDY

SEQ ID NO: 65 - DNA, 382 bp, synthetic construct
  misc_feature 1..382: note = MF3099
  source 1..382: mol_type = other DNA
  CDS 20..382
ggcccagccggccatggccgaggtccagctgcagcagcctggggctgagctggtgaggcctgggacttcagtgaagttgtcctgcaaggcttctggctacaccttcaccagctactggatgcactgggtaaagcagaggcctggacaaggccttgagtggatcggaattcttgatccttctgatagttatactacctacaatcaaaagttcaagggcaaggccacattaacagtagacacatcctccagcatagcctacatgcagctcagcagcctgacatctgaggactctgcgctctattactgtgcaagagggggagattacgacgagggaggtgctatggactactggggtcaaggaacctcggtcaccgtctccagt

SEQ ID NO: 66 - protein, 121 aa, synthetic construct
  REGION 1..121: note = Synthetic Construct; note = translation of SEQ ID NO:65
EVQLQQPGAELVRPGTSVKLSCKASGYTFTSYWMHWVKQRPGQGLEWIGILDPSDSYTTYNQKFKGKATLTVDTSSSIAYMQLSSLTSEDSALYYCARGGDYDEGGAMDYWGQGTSVTVSS

SEQ ID NO: 67 - protein, 5 aa, synthetic construct
  REGION 1..5: note = MF3099 CDR1
SYWMH

SEQ ID NO: 68 - protein, 17 aa, synthetic construct
  REGION 1..17: note = MF3099 CDR2
ILDPSDSYTTYNQKFKG

SEQ ID NO: 69 - protein, 12 aa, synthetic construct
  REGION 1..12: note = MF3099 CDR3
GGDYDEGGAMDY

SEQ ID NO: 70 - DNA, 391 bp, synthetic construct
  misc_feature 1..391: note = MF3307
  source 1..391: mol_type = other DNA
  CDS 20..391
ggcccagccggccatggcccaggtgcagctggtgcagtctggggctgaggtgaagaagcctggggcctcagtgaaggtctcctgcaaggcttctggatacaccttcaccggctactatatgcactgggtgcgacaggcccctggacaagggcttgagtggatgggatggatcaaccctaacagtggtggcacaaactatgcacagaagtttcagggcagggtcacgatgaccagggacacgtccatcagcacagcctacatggagctgagcaggctgagatctgacgacacggccgtgtattactgtgcaagaggttctcgtaaacgtctgtctaactacttcaacgcctttgattattggggccaaggtaccctggtcaccgtctccagt

SEQ ID NO: 71 - protein, 124 aa, synthetic construct
  REGION 1..124: note = Synthetic Construct; note = translation of SEQ ID NO:70
QVQLVQSGAEVKKPGASVKVSCKASGYTFTGYYMHWVRQAPGQGLEWMGWINPNSGGTNYAQKFQGRVTMTRDTSISTAYMELSRLRSDDTAVYYCARGSRKRLSNYFNAFDYWGQGTLVTVSS

SEQ ID NO: 72 - protein, 17 aa, synthetic construct
  REGION 1..17: note = MF3307 CDR2
WINPNSGGTNYAQKFQG

SEQ ID NO: 73 - protein, 15 aa, synthetic construct
  REGION 1..15: note = MF3307 CDR3
GSRKRLSNYFNAFDY

SEQ ID NO: 74 - protein, 95 aa, synthetic construct
  REGION 1..95: note = variable region of IGKV1-39
DIQMTQSPSSLSASVGDRVTITCRASQSISSYLNWYQQKPGKAPKLLIYAASSLQSGVPSRFSGSGSGTDFTLTISSLQPEDFATYYCQQSYSTP

SEQ ID NO: 75 - protein, 11 aa, synthetic construct
  REGION 1..11: note = IGKV1-39 CDR1
RASQSISSYLN

SEQ ID NO: 76 - protein, 7 aa, synthetic construct
  REGION 1..7: note = IGKV1-39 CDR2
AASSLQS

SEQ ID NO: 77 - protein, 9 aa, synthetic construct
  REGION 1..9: note = IGKV1-39 CDR3
QQSYSTPPT

SEQ ID NO: 78 - protein, 107 aa, synthetic construct
  REGION 1..107: note = IGKV1-39/jk1
DIQMTQSPSSLSASVGDRVTITCRASQSISSYLNWYQQKPGKAPKLLIYAASSLQSGVPSRFSGSGSGTDFTLTISSLQPEDFATYYCQQSYSTPPTFGQGTKVEIK

SEQ ID NO: 79 - protein, 214 aa, synthetic construct
  REGION 1..214: note = IGKV1-39/jk1 common light chain
DIQMTQSPSSLSASVGDRVTITCRASQSISSYLNWYQQKPGKAPKLLIYAASSLQSGVPSRFSGSGSGTDFTLTISSLQPEDFATYYCQQSYSTPPTFGQGTKVEIKRTVAAPSVFIFPPSDEQLKSGTASVVCLLNNFYPREAKVQWKVDNALQSGNSQESVTEQDSKDSTYSLSSTLTLSKADYEKHKVYACEVTHQGLSSPVTKSFNRGEC

SEQ ID NO: 80 - protein, 108 aa, synthetic construct
  REGION 1..108: note = IGKV1-39/jk5
DIQMTQSPSSLSASVGDRVTITCRASQSISSYLNWYQQKPGKAPKLLIYAASSLQSGVPSRFSGSGSGTDFTLTISSLQPEDFATYYCQQSYSTPPITFGQGTRLEIK

SEQ ID NO: 81 - protein, 450 aa, synthetic construct
  REGION 1..450: note = heavy chain for erbB-2 binding
QVQLVQSGAEVKKPGASVKLSCKASGYTFTAYYINWVRQAPGQGLEWIGRIYPGSGYTSYAQKFQGRATLTADESTSTAYMELSSLRSEDTAVYFCARPPVYYDSAWFAYWGQGTLVTVSSASTKGPSVFPLAPSSKSTSGGTAALGCLVKDYFPEPVTVSWNSGALTSGVHTFPAVLQSSGLYSLSSVVTVPSSSLGTQTYICNVNHKPSNTKVDKRVEPKSCDKTHTCPPCPAPELLGGPSVFLFPPKPKDTLMISRTPEVTCVVVDVSHEDPEVKFNWYVDGVEVHNAKTKPREEQYNSTYRVVSVLTVLHQDWLNGKEYKCKVSNKALPAPIEKTISKAKGQPREPQVYTDPPSREEMTKNQVSLTCEVKGFYPSDIAVEWESNGQPENNYKTTPPVLDSDGSFFLYSKLTVDKSRWQQGNVFSCSVMHEALHNHYTQKSLSLSPG

SEQ ID NO: 82 - protein, 453 aa, synthetic construct
  REGION 1..453: note = heavy chain for erbB-3 binding
QVQLVQSGAEVKKPGASVKVSCKASGYTFTGYYMHWVRQAPGQGLEWMGWINPNSGGTNYAQKFQGRVTMTRDTSISTAYMELSRLRSDDTAVYYCARDHGSRHFWSYWGFDYWGQGTLVTVSSASTKGPSVFPLAPSSKSTSGGTAALGCLVKDYFPEPVTVSWNSGALTSGVHTFPAVLQSSGLYSLSSVVTVPSSSLGTQTYICNVNHKPSNTKVDKRVEPKSCDKTHTCPPCPAPELLGGPSVFLFPPKPKDTLMISRTPEVTCVVVDVSHEDPEVKFNWYVDGVEVHNAKTKPREEQYNSTYRVVSVLTVLHQDWLNGKEYKCKVSNKALPAPIEKTISKAKGQPREPQVYTKPPSREEMTKNQVSLKCLVKGFYPSDIAVEWESNGQPENNYKTTPPVLDSDGSFFLYSKLTVDKSRWQQGNVFSCSVMHEALHNHYTQKSLSLSPG

SEQ ID NO: 83 - DNA, 379 bp, synthetic construct
  misc_feature 1..379: note = MF2889
  source 1..379: mol_type = other DNA
  CDS 20..379
ggcccagccggccatggccgaggtccagctgcagcagtctggagctgagctggtaaggcctgggacttcagtgaaggtgtcctgcaaggcttctggatacgccttcactaattatttgatagagtgggtaaagcagaggcctggccagggccttgagtggattggagtgatttatcctgaaggtggtggtactatctacaatgagaagttcaagggcaaggcaacactgactgcagacaaatcctccagcactgcctacatgcagctcagcggcctgacatctgaggactctgcggtctatttctgtgcaagaggagactatgattacaaatatgctatggactactggggtcaaggaacctcggtcaccgtctccagt

SEQ ID NO: 84 - protein, 120 aa, synthetic construct
  REGION 1..120: note = Synthetic Construct; note = translation of SEQ ID NO:83
EVQLQQSGAELVRPGTSVKVSCKASGYAFTNYLIEWVKQRPGQGLEWIGVIYPEGGGTIYNEKFKGKATLTADKSSSTAYMQLSGLTSEDSAVYFCARGDYDYKYAMDYWGQGTSVTVSS

SEQ ID NO: 85 - protein, 5 aa, synthetic construct
  REGION 1..5: note = MF2889 CDR1
NYLIE

SEQ ID NO: 86 - protein, 17 aa, synthetic construct
  REGION 1..17: note = MF2889 CDR2
VIYPEGGGTIYNEKFKG

SEQ ID NO: 87 - protein, 11 aa, synthetic construct
  REGION 1..11: note = MF2889 CDR3
GDYDYKYAMDY

SEQ ID NO: 88 - DNA, 370 bp, synthetic construct
  misc_feature 1..370: note = MF2913
  source 1..370: mol_type = other DNA
  CDS 20..370
ggcccagccggccatggccgaggtcaagctgcagcagtctggacctgagctggtgaagcctggcgcttcagtgaagatatcctgcaaggcttctggttactcattcactgactacaaaatggactgggtgaagcagagccatggaaagagcctcgaatggattggaaatattaatcctaacagtggtggtgttatctacaaccagaagttcaggggcaaggtcacattgactgttgacaggtcctccagcgcagcctacatggagctccgcagcctgacatctgaggacactgcagtctattattgttcaagaggactgtgggatgctatggactcctggggtcaaggaacctcggtcaccgtctccagt

SEQ ID NO: 89 - protein, 117 aa, synthetic construct
  REGION 1..117: note = Synthetic Construct; note = translation of SEQ ID NO:88
EVKLQQSGPELVKPGASVKISCKASGYSFTDYKMDWVKQSHGKSLEWIGNINPNSGGVIYNQKFRGKVTLTVDRSSSAAYMELRSLTSEDTAVYYCSRGLWDAMDSWGQGTSVTVSS

SEQ ID NO: 90 - protein, 16 aa, synthetic construct
  REGION 1..16: note = MF2913 CDR1
DYKMDWVKQSHGKSLE

SEQ ID NO: 91 - protein, 6 aa, synthetic construct
  REGION 1..6: note = MF2913 CDR2
NQKFRG

SEQ ID NO: 92 - protein, 8 aa, synthetic construct
  REGION 1..8: note = MF2913 CDR3
GLWDAMDS

SEQ ID NO: 93 - DNA, 382 bp, synthetic construct
  misc_feature 1..382: note = MF1847
  source 1..382: mol_type = other DNA
  CDS 20..382
ggcccagccggccatggcccaggtgcagctggtggagtctgggggaggcgtggtccagcctgggaggtccctgagactctcctgtgcagcctctggattcaccttcagtagctatggcatgcactgggtccgccaggctccaggcaaggggctggagtgggtggcagttatatcatatgatggaagtaataaatactatgcagactccgtgaagggccgattcaccatctccagagacaattccaagaacacgctgtatctgcaaatgaacagcctgagagctgaggacacggccgtgtattactgtgcaaaaggttggtggcatccgctgctgtctggctttgattattggggccaaggtaccctggtcaccgtctccagt

SEQ ID NO: 94 - protein, 121 aa, synthetic construct
  REGION 1..121: note = Synthetic Construct; note = translation of SEQ ID NO:93
QVQLVESGGGVVQPGRSLRLSCAASGFTFSSYGMHWVRQAPGKGLEWVAVISYDGSNKYYADSVKGRFTISRDNSKNTLYLQMNSLRAEDTAVYYCAKGWWHPLLSGFDYWGQGTLVTVSS

SEQ ID NO: 95 - protein, 5 aa, synthetic construct
  REGION 1..5: note = MF1847 CDR1
SYGMH

SEQ ID NO: 96 - protein, 17 aa, synthetic construct
  REGION 1..17: note = MF1847 CDR2
VISYDGSNKYYADSVKG

SEQ ID NO: 97 - protein, 12 aa, synthetic construct
  REGION 1..12: note = MF1847 CDR3
GWWHPLLSGFDY

SEQ ID NO: 98 - DNA, 370 bp, synthetic construct
  misc_feature 1..370: note = MF3001
  source 1..370: mol_type = other DNA
  CDS 20..370
ggcccagccggccatggccgaggtccagctgcagcagtctggggctgaactggcaaaacctggggcctcagtgaagctgtcctgcaagacttctggctacaactttcctatctactggatgcactgggtaaaacagaggcctggacggggtctggaatggattggatacattaatcctagtactggttatattaagaacaatcagaagttcaaggacaaggccaccttgactgcagacaaatcctccaacacagcctacatgcagctgaacagcctgacatatgaggactctgcagtctattactgtacaagagaagggataactgggtttacttactggggccaagggactctggtcaccgtctccagt

SEQ ID NO: 99 - protein, 117 aa, synthetic construct
  REGION 1..117: note = Synthetic Construct; note = translation of SEQ ID NO:98
EVQLQQSGAELAKPGASVKLSCKTSGYNFPIYWMHWVKQRPGRGLEWIGYINPSTGYIKNNQKFKDKATLTADKSSNTAYMQLNSLTYEDSAVYYCTREGITGFTYWGQGTLVTVSS

SEQ ID NO: 100 - protein, 16 aa, synthetic construct
  REGION 1..16: note = MF3001 CDR1
IYWMHWVKQRPGRGLE

SEQ ID NO: 101 - protein, 6 aa, synthetic construct
  REGION 1..6: note = MF3001 CDR2
NQKFKD

SEQ ID NO: 102 - protein, 8 aa, synthetic construct
  REGION 1..8: note = MF3001 CDR3
EGITGFTY

SEQ ID NO: 103 - DNA, 385 bp, synthetic construct
  misc_feature 1..385: note = MF1898
  source 1..385: mol_type = other DNA
  CDS 20..385
ggcccagccggccatggcccaggtgcagctggtggagtctgggggaggcgtggtccagcctgggaggtccctgagactctcctgtgcagcctctggattcaccttcagtagctatggcatgcactgggtccgccaggctccaggcaaggggctggagtgggtggcagttatatcatatgatggaagtaataaatactatgcagactccgtgaagggccgattcaccatctccagagacaattccaagaacacgctgtatctgcaaatgaacagcctgagagctgaggacacggccgtgtattactgtgcaaaagatggtttccgtcgtactactctgtctggctttgattattggggccaaggtaccctggtcaccgtctccagt

SEQ ID NO: 104 - protein, 122 aa, synthetic construct
  REGION 1..122: note = Synthetic Construct; note = translation of SEQ ID NO:103
QVQLVESGGGVVQPGRSLRLSCAASGFTFSSYGMHWVRQAPGKGLEWVAVISYDGSNKYYADSVKGRFTISRDNSKNTLYLQMNSLRAEDTAVYYCAKDGFRRTTLSGFDYWGQGTLVTVSS

SEQ ID NO: 105 - protein, 13 aa, synthetic construct
  REGION 1..13: note = MF1898 CDR3
DGFRRTTLSGFDY

SEQ ID NO: 106 - DNA, 379 bp, synthetic construct
  misc_feature 1..379: note = MF3003
  source 1..379: mol_type = other DNA
  CDS 20..379
ggcccagccggccatggcccaggtgcagctgaagcagtctggacctgagctggtgaagcctggggcctcagtgaagatttcctgcaaggcttctggcgacgcattcagttactcctggatgaactgggtgaagcagaggcctggaaagggtcttgagtggattggacggatttatcctggagatggagatattaactacaatgggaagttcaagggcaaggccacactgactgcagacaaatcctccagcacagcccacctgcaactcaacagcctgacatctgaggactctgcggtctacttctgtgcaagaggacagctcggactagaggcctggtttgcttattggggccaggggactctggtcaccgtctccagt

SEQ ID NO: 107 - protein, 120 aa, synthetic construct
  REGION 1..120: note = Synthetic Construct; note = translation of SEQ ID NO:106
QVQLKQSGPELVKPGASVKISCKASGDAFSYSWMNWVKQRPGKGLEWIGRIYPGDGDINYNGKFKGKATLTADKSSSTAHLQLNSLTSEDSAVYFCARGQLGLEAWFAYWGQGTLVTVSS

SEQ ID NO: 108 - protein, 16 aa, synthetic construct
  REGION 1..16: note = MF3003 CDR1
YSWMNWVKQRPGKGLE

SEQ ID NO: 109 - protein, 6 aa, synthetic construct
  REGION 1..6: note = MF3003 CDR2
NGKFKG

SEQ ID NO: 110 - protein, 11 aa, synthetic construct
  REGION 1..11: note = MF3003 CDR3
GQLGLEAWFAY

SEQ ID NO: 111 - DNA, 391 bp, synthetic construct
  misc_feature 1..391: note = MF6058
  source 1..391: mol_type = other DNA
  CDS 20..391
ggcccagccggccatggcccaggtgcagctggtgcagtctggggctgacgtgaagaagcctggggcctcagtgaaggtcacgtgcaaggcttctggatacaccttcaccggctactatatgcactgggtgcgacaggcccctggacaagctcttgagtggatgggatggatcaaccctcaaagtggtggcacaaactatgcaaagaagtttcagggcagggtctctatgaccagggagacgtccacaagcacagcctacatgcagctgagcaggctgagatctgacgacacggctacgtattactgtgcaagagatcatggttctcgtcatttctggtcttactggggctttgattattggggccaaggtaccctggtcaccgtctccagt

SEQ ID NO: 112 - protein, 124 aa, synthetic construct
  REGION 1..124: note = Synthetic Construct; note = translation of SEQ ID NO:111
QVQLVQSGADVKKPGASVKVTCKASGYTFTGYYMHWVRQAPGQALEWMGWINPQSGGTNYAKKFQGRVSMTRETSTSTAYMQLSRLRSDDTATYYCARDHGSRHFWSYWGFDYWGQGTLVTVSS

SEQ ID NO: 113 - protein, 17 aa, synthetic construct
  REGION 1..17: note = MF6058 CDR2
WINPQSGGTNYAKKFQG

SEQ ID NO: 114 - protein, 15 aa, synthetic construct
  REGION 1..15: note = MF6058 CDR3
DHGSRHFWSYWGFDY

SEQ ID NO: 115 - DNA, 391 bp, synthetic construct
  misc_feature 1..391: note = MF6061
  source 1..391: mol_type = other DNA
  CDS 20..391
ggcccagccggccatggcccaggtgcagctggtgcagtctggggctgaggtgaagaagcctggggcctcagtgaaggtctcctgcaaggcttctggatacaccttcaccggctactatatgcactgggtgcgacaggcccctggacaagggcttgagtggatgggatggatcaaccctcagagtggtggcacaaactatgcacagaagtttaagggcagggtcacgatgaccagggacacgtccaccagcacagcctacatggagctgagcaggctgagatctgacgacacggctgtgtattactgtgcaagagatcatggttctcgtcatttctggtcttactggggctttgattattggggccaaggtaccctggtcaccgtctccagt

SEQ ID NO: 116 - protein, 124 aa, synthetic construct
  REGION 1..124: note = Synthetic Construct; note = translation of SEQ ID NO:115
QVQLVQSGAEVKKPGASVKVSCKASGYTFTGYYMHWVRQAPGQGLEWMGWINPQSGGTNYAQKFKGRVTMTRDTSTSTAYMELSRLRSDDTAVYYCARDHGSRHFWSYWGFDYWGQGTLVTVSS

SEQ ID NO: 117 - protein, 17 aa, synthetic construct
  REGION 1..17: note = MF6061 CDR2
WINPQSGGTNYAQKFKG

SEQ ID NO: 118 - DNA, 391 bp, synthetic construct
  misc_feature 1..391: note = MF6065
  source 1..391: mol_type = other DNA
  CDS 20..391
ggcccagccggccatggcccaggtgcagctggtgcagtctggggctgaggtgaagaagcctggggcctcagtgaaggtctcctgcaaggcttctggatacaccttcacctcttactatatgcactgggtgcgacaggcccctggacaagggcttgagtggatgggatggatcaaccctcaggggggttctacaaactatgcacagaagtttcagggcagggtcacgatgaccagggacacgtccaccagcacagtgtacatggagctgagcaggctgagatctgaggacacggctgtgtattactgtgcaagagatcatggttctcgtcatttctggtcttactggggctttgattattggggccaaggtaccctggtcaccgtctccagt

SEQ ID NO: 119 - protein, 124 aa, synthetic construct
  REGION 1..124: note = Synthetic Construct; note = translation of SEQ ID NO:118
QVQLVQSGAEVKKPGASVKVSCKASGYTFTSYYMHWVRQAPGQGLEWMGWINPQGGSTNYAQKFQGRVTMTRDTSTSTVYMELSRLRSEDTAVYYCARDHGSRHFWSYWGFDYWGQGTLVTVSS

SEQ ID NO: 120 - protein, 5 aa, synthetic construct
  REGION 1..5: note = MF6065 CDR1
SYYMH

SEQ ID NO: 121 - protein, 17 aa, synthetic construct
  REGION 1..17: note = MF6065 CDR2
WINPQGGSTNYAQKFQG

SEQ ID NO: 122 - protein, 124 aa, synthetic construct
  REGION 1..124: note = MF6055
QVQLVQSGADVKKPGASVKVSCKASGYTFTGYYMHWVRQAPGQALEWMGWINPSSGGTNYAKKFQGRVTMTRETSTSTAYMELSRLRSDDTATYYCARDHGSRHFWSYWGFDYWGQGTLVTVSS

SEQ ID NO: 123 - protein, 124 aa, synthetic construct
  REGION 1..124: note = MF6056
QVQLVQSGADVKKPGASVKVTCKASGYTFTGYYMHWVRQAPGQALEWMGWINPSSGGTNYAKKFQGRVSMTRETSTSTAYMQLSRLRSDDTATYYCARDHGSRHFWSYWGFDYWGQGTLVTVSS

SEQ ID NO: 124 - protein, 124 aa, synthetic construct
  REGION 1..124: note = MF6057
QVQLVQSGADVKKPGASVKVTCKASGYTFTGYYMHWVRQAPGQGLEWMGWINPQSGGTNYAQKFQGRVTMTRDTSISTAYMQLSRLRSDDTAVYYCARDHGSRHFWSYWGFDYWGQGTLVTVSS

SEQ ID NO: 125 - protein, 124 aa, synthetic construct; identical to SEQ ID NO: 112
  REGION 1..124: note = MF6058

SEQ ID NO: 126 - protein, 124 aa, synthetic construct
  REGION 1..124: note = MF6059
QVQLVQSGAEVKKPGASVKVSCKASGYTFTGYYMHWVRQAPGQGLEWMGWINPGSGSTNYAQKFQGRVTMTRDTSISTAYMELSRLRSDDTAVYYCARDHGSRHFWSYWGFDYWGQGTLVTVSS

SEQ ID NO: 127 - protein, 124 aa, synthetic construct
  REGION 1..124: note = MF6060
QVQLVQSGADVKKPGASVKVSCKASGYTFTGYYMHWVRQAPGQALEWMGWINPQSGGTNYAKKFQGRVTMTRETSTSTAYMELSRLRSDDTATYYCARDHGSRHFWSYWGFDYWGQGTLVTVSS

SEQ ID NO: 128 - protein, 124 aa, synthetic construct; identical to SEQ ID NO: 116
  REGION 1..124: note = MF6061

SEQ ID NO: 129 - protein, 124 aa, synthetic construct
  REGION 1..124: note = MF6062
QVQLVQSGAEVKKPGASVKVSCKASGYTFTGYYMHWVRQAPGQGLEWMGWINPGSGSTNYAQKFQGRVTMTRDTSTSTAYMELSRLRSDDTAVYYCARDHGSRHFWSYWGFDYWGQGTLVTVSS

SEQ ID NO: 130 - protein, 124 aa, synthetic construct
  REGION 1..124: note = MF6063
QVQLVQSGAEVKKPGASVKVSCKASGYTFTGYYMHWVRQAPGQGLEWMGWINPQSGGTNYAKKFQGRVTMTRDTSTSTAYMELSRLRSDDTAVYYCARDHGSRHFWSYWGFDYWGQGTLVTVSS

SEQ ID NO: 131 - protein, 124 aa, synthetic construct
  REGION 1..124: note = MF6064
QVQLVQSGAEVKKPGASVKVSCKASGYTFTGYYMHWVRQAPGKGLEWMGWINPQSGGTNYAQKFQGRVTMTRDTSTSTAYMELSRLRSDDTAVYYCARDHGSRHFWSYWGFDYWGQGTLVTVSS

SEQ ID NO: 132 - protein, 124 aa, synthetic construct; identical to SEQ ID NO: 119
  REGION 1..124: note = MF6065

SEQ ID NO: 133 - protein, 124 aa, synthetic construct
  REGION 1..124: note = MF6066
QVQLVQSGAEVKKPGASVKVSCKASGYTFTGYYMHWVRQAPGQGLEWMGWINPQSGSTNYAQKFQGRVTMTRDTSTSTAYMELSSLRSEDTAVYYCARDHGSRHFWSYWGFDYWGQGTLVTVSS

SEQ ID NO: 134 - protein, 124 aa, synthetic construct
  REGION 1..124: note = MF6067
QVQLVQSGAEVKKPGASVKVSCKASGYTFTGYYMHWVRQAPGQGLEWMGWINPQSGGTNYAQKFQGRVTMTRDTSTSTAVMELSSLRSDDTAVYYCARDHGSRHFWSYWGFDYWGQGTLVTVSS

SEQ ID NO: 135 - protein, 124 aa, synthetic construct
  REGION 1..124: note = MF6068
QVQLVQSGAEVKKPGASVKVSCKASGYTFTGYYMHWVRQAPGQGLEWMGWINPQSGGTNYAQKFQGRVTMTRDTSTSTAYMELSRLRSDDTAVYYCARDHGSRHFWSYWGFDYWGQGTLVTVSS

SEQ ID NO: 136 - protein, 124 aa, synthetic construct
  REGION 1..124: note = MF6069
QVQLVQSGAEVKKPGASVKVSCKASGYTFTGYYMHWVRQAPGQGLEWMGWINPQSGGTNYAQKFQGRVTMTRDTSISTAYMELSRLRSDDTAVYYCARDHGSRHFWSYWGFDYWGQGTLVTVSS

SEQ ID NO: 137 - protein, 124 aa, synthetic construct
  REGION 1..124: note = MF6070
QVQLVQSGAEVKKPGASVKVSCKASGYTFTSYYMHWVRQAPGQGLEWMGWINPSGGSTNYAQKFQGRVTMTRDTSTSTVYMELSRLRSEDTAVYYCARDHGSRHFWSYWGFDYWGQGTLVTVSS

SEQ ID NO: 138 - protein, 124 aa, synthetic construct
  REGION 1..124: note = MF6071
QVQLVQSGAEVKKPGASVKVSCKASGYTFTGYYMHWVRQAPGQGLEWMGWINPSSGSTNYAQKFQGRVTMTRDTSTSTAYMELSSLRSEDTAVYYCARDHGSRHFWSYWGFDYWGQGTLVTVSS

SEQ ID NO: 139 - protein, 124 aa, synthetic construct
  REGION 1..124: note = MF6072
QVQLVQSGAEVKKPGASVKVSCKASGYTFTGYYMHWVRQAPGQGLEWMGWINPSSGGTNYAQKFQGRVTMTRDTSTSTVYMELSSLRSDDTAVYYCARDHGSRHFWSYWGFDYWGQGTLVTVSS

SEQ ID NO: 140 - protein, 124 aa, synthetic construct
  REGION 1..124: note = MF6073
QVQLVQSGAEVKKPGASVKVSCKASGYTFTGYYMHWVRQAPGQGLEWMGWINPSSGGTNYAQKFQGRVTMTRDTSTSTAYMELSRLRSDDTAVYYCARDHGSRHFWSYWGFDYWGQGTLVTVSS

SEQ ID NO: 141 - protein, 124 aa, synthetic construct
  REGION 1..124: note = MF6074
QVQLVQSGAEVKKPGASVKVSCKASGYTFTGYYMHWVRQAPGQGLEWMGWINPSSGGTNYAQKFQGRVTMTRDTSISTAYMELSRLRSDDTAVYYCARDHGSRHFWSYWGFDYWGQGTLVTVSS